European Patent Specification EP 3 524 261 B1, published December 13, 2023. Title: METHODS FOR TREATING DIABETES AND REDUCING BODY WEIGHT. Applicant: Amylin Pharmaceuticals, Inc. Fineman, Mark MacConell, Leigh Taylor, Kristin. The sequence listing filed with the application follows.

SEQUENCE LISTING (142 sequences)

SEQ ID NO: 1 - protein, 39 aa, Heloderma horridum
  MOD_RES (39)..(39): AMIDATION
HGEGTFTSDLSKQMEEEAVRLFIEWLKNGGPSSGAPPPS

SEQ ID NO: 2 - protein, 39 aa, Heloderma suspectum
  MOD_RES (39)..(39): AMIDATION
HSDGTFTSDLSKQMEEEAVRLFIEWLKNGGPSSGAPPPS

SEQ ID NO: 3 - protein, 30 aa, Homo sapiens
  MOD_RES (30)..(30): AMIDATION
HAEGTFTSDVSSYLEGQAAKEFIAWLVKGR

SEQ ID NO: 4 - protein, 31 aa, Heloderma horridum
  MOD_RES (31)..(31): AMIDATION
DLSKQMEEEAVRLFIEWLKNGGPSSGAPPPS

SEQ ID NO: 5 - protein, 38 aa, Heloderma horridum
HSDATFTAEYSKLLAKLALQKYLESILGSSTSPRPPSS

SEQ ID NO: 6 - protein, 37 aa, Heloderma horridum
HSDATFTAEYSKLLAKLALQKYLESILGSSTSPRPPS

SEQ ID NO: 7 - protein, 35 aa, Heloderma suspectum
  MOD_RES (35)..(35): AMIDATION
HSDAIFTEEYSKLLAKLALQKYLASILGSRTSPPP

SEQ ID NO: 8 - protein, 35 aa, Artificial Sequence
  Exendin analog
  MOD_RES (35)..(35): AMIDATION
HSDAIFTQQYSKLLAKLALQKYLASILGSRTSPPP

SEQ ID NO: 9 - protein, 30 aa, Artificial Sequence
  Exendin analog
HGEGTFTSDLSKQMEEEAVRLFIEWLKNGG

SEQ ID NO: 10 - protein, 30 aa, Artificial Sequence; identical to SEQ ID NO: 9
  Exendin analog
  MOD_RES (30)..(30): AMIDATION

SEQ ID NO: 11 - protein, 28 aa, Artificial Sequence
  Exendin analog
  MOD_RES (28)..(28): AMIDATION
HGEGTFTSDLSKQMEEEAVRLFIEWLKN

SEQ ID NO: 12 - protein, 39 aa, Artificial Sequence
  Exendin analog
  MOD_RES (39)..(39): AMIDATION
HGEGTFTSDLSKQLEEEAVRLFIEFLKNGGPSSGAPPPS

SEQ ID NO: 13 - protein, 28 aa, Artificial Sequence
  Exendin analog
  MOD_RES (28)..(28): AMIDATION
HGEGTFTSDLSKQLEEEAVRLFIEFLKN

SEQ ID NO: 14 - protein, 28 aa, Artificial Sequence
  MOD_RES (28)..(28): AMIDATION
  Exendin analog
HGEGTFTSDLSKQLEEEAVRLAIEFLKN

SEQ ID NO: 15 - protein, 38 aa, Artificial Sequence
  Exendin analog
  MISC_FEATURE (1)..(1): His, Arg, or Tyr
  MISC_FEATURE (2)..(2): Ser, Gly, Ala or Thr
  MISC_FEATURE (3)..(3): Ala, Asp or Glu
  MISC_FEATURE (4)..(4): Ala or Thr
  MISC_FEATURE (5)..(5): Ala or Thr
  MISC_FEATURE (6)..(6): Ala, Phe, Tyr or naphthylalanine
  MISC_FEATURE (7)..(7): Thr or Ser
  MISC_FEATURE (8)..(8): Ala, Ser or Thr
  MISC_FEATURE (9)..(9): Asp or Glu
  MISC_FEATURE (10)..(10): Ala, Leu, Ile, Val, pentylglycine or Met
  MISC_FEATURE (11)..(11): Ala or Ser
  MISC_FEATURE (12)..(12): Ala or Lys
  MISC_FEATURE (13)..(13): Ala or Gln
  MISC_FEATURE (14)..(14): Ala, Leu, Ile, pentylglycine, Val or Met
  MISC_FEATURE (15)..(15): Ala or Glu
  MISC_FEATURE (16)..(16): Ala or Glu
  MISC_FEATURE (17)..(17): Ala or Glu
  MISC_FEATURE (19)..(19): Ala or Val
  MISC_FEATURE (20)..(20): Ala or Arg
  MISC_FEATURE (21)..(21): Ala or Leu
  MISC_FEATURE (22)..(22): Ala, Phe, Tyr or naphthylalanine
  MISC_FEATURE (23)..(23): Ile, Val, Leu, pentylglycine, tert-butylglycine or Met
  MISC_FEATURE (24)..(24): Ala Glu or Asp
  MISC_FEATURE (25)..(25): Ala, Trp, Phe, Tyr or naphthylalanine
  MISC_FEATURE (26)..(26): Ala or Leu
  MISC_FEATURE (27)..(27): Ala or Lys
  MISC_FEATURE (28)..(28): Ala or Asn and is optionally amidated
  MISC_FEATURE (29)..(29): Gly or absent and if present optionally amidated
  MISC_FEATURE (30)..(30): Gly or absent and if present optionally amidated
  MISC_FEATURE (31)..(31): Pro, homoproline, 3Hyp, 4Hyp, Thioproline, N-alkylglycine, N-alkylpentylglycine, N-alkylalanine or absent and if present optionally amidated
  MISC_FEATURE (32)..(32): Ser or absent and if present optionally amidated
  MISC_FEATURE (33)..(33): Ser or absent and if present optionally amidated
  MISC_FEATURE (34)..(34): Gly or absent and if present optionally amidated
  MISC_FEATURE (35)..(35): Ala or absent and if present optionally amidated
  MISC_FEATURE (36)..(38): Pro, homoproline, 3Hyp, 4Hyp, Thioproline, N-alkylglycine, N-alkylpentylglycine, N-alkylalanine or absent and if present optionally amidated
XXXGXXXXXXXXXXXXXAXXXXXXXXXXGGXSSGAXXX

SEQ ID NO: 16 - protein, 39 aa, Artificial Sequence
  Exendin analog
  MISC_FEATURE (1)..(1): His, Arg, Tyr, Ala, Norval, Val or Norleu
  MISC_FEATURE (2)..(2): Ser, Gly, Ala or Thr
  MISC_FEATURE (3)..(3): Ala, Asp or Glu
  MISC_FEATURE (4)..(4): Ala, Norval, Val, Norleu or Gly
  MISC_FEATURE (5)..(5): Ala or Thr
  MISC_FEATURE (6)..(6): Ala, Phe, Tyr or naphthylalanine
  MISC_FEATURE (7)..(7): Thr or Ser
  MISC_FEATURE (8)..(8): Ala, Ser or Thr
  MISC_FEATURE (9)..(9): Ala, Norva, Val, Norleu, Asp or Glu
  MISC_FEATURE (10)..(10): Ala, Leu, Ile, Val, pentylglycine or Met
  MISC_FEATURE (11)..(11): Ala or Ser
  MISC_FEATURE (12)..(12): Ala or Lys
  MISC_FEATURE (13)..(13): Ala or Gln
  MISC_FEATURE (14)..(14): Ala, Leu, Ile, pentylglycine, Val or Met
  MISC_FEATURE (15)..(17): Ala or Glu
  MISC_FEATURE (19)..(19): Ala or Val
  MISC_FEATURE (20)..(20): Ala or Arg
  MISC_FEATURE (21)..(21): Ala or Leu
  MISC_FEATURE (22)..(22): Phe, Tyr or naphthylalanine
  MISC_FEATURE (23)..(23): Ile, Val, Keu, pentylglycine, tert-butylglycine or Met
  MISC_FEATURE (24)..(24): Ala, Glu or Asp
  MISC_FEATURE (25)..(25): Ala, Trp, Phe, Tyr or naphthylalanine
  MISC_FEATURE (26)..(26): Ala or Leu
  MISC_FEATURE (27)..(27): Ala or Lys
  MISC_FEATURE (28)..(28): Ala or Asn and optionally amidated
  MISC_FEATURE (29)..(30): Gly or absent and if present optionally amidated
  MISC_FEATURE (31)..(31): Pro, homoproline, 3Hyp, 4Hyp, thioproline, N-alkylglycine, N-alkylpentylglycine or N-alkylalanine or absent and if present optionally amidated
  MISC_FEATURE (32)..(33): Ser or absent and if present optionally amidated
  MISC_FEATURE (34)..(34): Gly or absent and if present optionally amidated
  MISC_FEATURE (35)..(35): Ser or absent and if present optionally amidated
  MISC_FEATURE (36)..(38): Pro, homoproline, 3Hyp, 4Hyp, thioproline, N-alkylglycine, N-alkylpentylglycine or N-alkylalanine or absent and if present optionally amidated
  MISC_FEATURE (39)..(39): Ser, Tyr or absent and if present optionally amidated
XXXXXXXXXXXXXXXXXAXXXXXXXXXXGGXSSGAXXXX

SEQ ID NO: 17 - protein, 38 aa, Artificial Sequence; identical to SEQ ID NO: 15
  Exendin analog
  MISC_FEATURE (1)..(1): His or Arg
  MISC_FEATURE (2)..(2): Gly or Ala
  MISC_FEATURE (3)..(3): Ala, Asp or Glu
  MISC_FEATURE (5)..(5): Ala or Thr
  MISC_FEATURE (6)..(6): Ala, Phe or naphthylalanine
  MISC_FEATURE (7)..(7): Thr or Ser
  MISC_FEATURE (8)..(8): Ala, Ser or Thr
  MISC_FEATURE (9)..(9): Asp or Glu
  MISC_FEATURE (10)..(10): Ala, Leu or pentylglycine
  MISC_FEATURE (11)..(11): Ala or Ser
  MISC_FEATURE (12)..(12): Ala or Lys
  MISC_FEATURE (13)..(13): Ala or Gln
  MISC_FEATURE (14)..(14): Ala, Leu or pentylglycine
  MISC_FEATURE (15)..(17): Ala or Glu
  MISC_FEATURE (19)..(19): Ala or Val
  MISC_FEATURE (20)..(20): Ala or Arg
  MISC_FEATURE (21)..(21): Ala or Leu
  MISC_FEATURE (22)..(22): Phe or napthylalanine
  MISC_FEATURE (23)..(23): Ile, Val or tert-butylglycine
  MISC_FEATURE (24)..(24): Ala, Glu or Asp
  MISC_FEATURE (25)..(25): Ala, Trp or Phe
  MISC_FEATURE (26)..(26): Ala or Leu
  MISC_FEATURE (27)..(27): Ala or Lys
  MISC_FEATURE (28)..(28): Ala or Asn and optionally amidated
  MISC_FEATURE (29)..(30): Gly or absent and if present optionally amidated
  MISC_FEATURE (31)..(31): Pro, homoproline, thioproline N-methylalanine or absent and if present optionally amidated
  MISC_FEATURE (32)..(33): Ser or absent and if present optionally amidated
  MISC_FEATURE (34)..(34): Gly or absent and if present optionally amidated
  MISC_FEATURE (35)..(35): Ala or absent and if present optionally amidated
  MISC_FEATURE (36)..(38): Pro, homoproline, thioproline N-methylalanine or absent and if present optionally amidated

SEQ ID NO: 18 - protein, 39 aa, Artificial Sequence
  Exendin analog
  MISC_FEATURE (1)..(1): His or Ala
  MISC_FEATURE (2)..(2): Gly or Ala
  MISC_FEATURE (3)..(3): Ala, Asp or Glu
  MISC_FEATURE (4)..(4): Ala or Gly
  MISC_FEATURE (5)..(5): Ala or Thr
  MISC_FEATURE (6)..(6): Ala, Phe or naphthylalanine
  MISC_FEATURE (7)..(7): Thr or Ser
  MISC_FEATURE (8)..(8): Ala, Ser or Thr
  MISC_FEATURE (9)..(9): Ala, Asp or Glu
  MISC_FEATURE (10)..(10): Ala, Leu or pentylglycine
  MISC_FEATURE (11)..(11): Ala or Ser
  MISC_FEATURE (12)..(12): Ala or Lys
  MISC_FEATURE (13)..(13): Ala or Gln
  MISC_FEATURE (14)..(14): Ala, Leu, Met or pentylglycine
  MISC_FEATURE (15)..(17): Ala or Glu
  MISC_FEATURE (19)..(19): Ala or Val
  MISC_FEATURE (20)..(20): Ala or Arg
  MISC_FEATURE (21)..(21): Ala or Leu
  MISC_FEATURE (22)..(22): Phe or naphthylalanine
  MISC_FEATURE (23)..(23): Ile, Val or tert-butylglycine
  MISC_FEATURE (24)..(24): Ala or Glu or Asp
  MISC_FEATURE (25)..(25): Ala, Trp or Phe
  MISC_FEATURE (26)..(26): Ala or Leu
  MISC_FEATURE (27)..(27): Ala or Lys
  MISC_FEATURE (28)..(28): Ala or Asn and optionally amidated
  MISC_FEATURE (29)..(30): Gly or absent and if present optionally amidated
  MISC_FEATURE (31)..(31): Pro, homoproline, thioproline, N-methylalanine or absent and if present optionally amidated
  MISC_FEATURE (32)..(33): Ser or absent and if present optionally amidated
  MISC_FEATURE (34)..(34): Gly or absent and if present optionally amidated
  MISC_FEATURE (35)..(35): Ala or absent and if present optionally amidated
  MISC_FEATURE (36)..(38): Pro, homoproline, thioproline, N-methylalanine or absent and if present optionally amidated
  MISC_FEATURE (39)..(39): Ser or absent and if present optionally amidated
XXXXXXXXXXXXXXXXXAXXXXXXXXXXGGXSSGAXXXS

SEQ ID NO: 19 - protein, 38 aa, Artificial Sequence; identical to SEQ ID NO: 15
  Exendin analog
  MISC_FEATURE (1)..(1): His, Arg, Tyr or imidazopropionyl
  MISC_FEATURE (2)..(2): Ser, Gly, Ala or Thr
  MISC_FEATURE (3)..(3): Ala, Asp or Glu
  MISC_FEATURE (5)..(5): Ala or Thr
  MISC_FEATURE (6)..(6): Ala, Phe, Tyr or naphthylalanine
  MISC_FEATURE (7)..(7): Thr or Ser
  MISC_FEATURE (8)..(8): Ala, Ser or Thr
  MISC_FEATURE (9)..(9): Asp or Glu
  MISC_FEATURE (10)..(10): Ala, Leu, Ile, Val, pentylglycine or Met
  MISC_FEATURE (11)..(11): Ala or Ser
  MISC_FEATURE (12)..(12): Ala or Lys
  MISC_FEATURE (13)..(13): Ala or Gln
  MISC_FEATURE (14)..(14): Ala, Leu, Ile, pentylglycine, Val or Met
  MISC_FEATURE (15)..(17): Ala or Glu
  MISC_FEATURE (19)..(19): Ala or Val
  MISC_FEATURE (20)..(20): Ala or Arg
  MISC_FEATURE (21)..(21): Ala, Leu or Lys-NH-R where R is Lys, Arg, C1-C10 straight chain or branched alkanoyl or cycloalkylalkanoyl
  MISC_FEATURE (22)..(22): Phe, Tyr or naphthylalanine
  MISC_FEATURE (23)..(23): Ile, Val, Leu, pentylglycine, tert-butylglycine or Met
  MISC_FEATURE (24)..(24): Ala, Glu or Asp
  MISC_FEATURE (25)..(25): Ala, Trp, Phe, Tyr or naphthylalanine
  MISC_FEATURE (26)..(26): Ala or Leu
  MISC_FEATURE (27)..(27): Lys, Asn, Ala or Lys-NH-R where R is Lys, Arg, C1-C10 straight chain or branched alkanoyl or cycloalkylalkanoyl
  MISC_FEATURE (28)..(28): Lys, Asn, Ala or Lys-NH-R where R is Lys, Arg, C1-C10 straight chain or branched alkanoyl or cycloalkylalkanoyl and is optionally amidated
  MISC_FEATURE (29)..(30): Gly or absent and if present optionally amidated
  MISC_FEATURE (31)..(31): Pro, homoproline, 3Hyp, 4Hyp, thioproline, N-alkylglycine, N-alkylpentylglycine, N-alkylalanine or absent and if present is optionally amidated
  MISC_FEATURE (32)..(33): Ser or absent and if present optionally amidated
  MISC_FEATURE (34)..(34): Gly or absent and if present optionally amidated
  MISC_FEATURE (35)..(35): Ala or absent and if present optionally amidated
  MISC_FEATURE (36)..(38): Pro, homoproline, 3Hyp, 4Hyp, thioproline, N-alkylglycine, N-alkylpentylglycine, N-alkylalanine or absent and if present is optionally amidated

SEQ ID NO: 20 - protein, 39 aa, Artificial Sequence; identical to SEQ ID NO: 16
  Exendin analog
  MISC_FEATURE (1)..(1): His, Arg, Tyr, Ala, Norval, Val Norleu or 4-imidazopropionyl
  MISC_FEATURE (2)..(2): Ser, Gly, Ala or Thr
  MISC_FEATURE (3)..(3): Ala, Asp or Glu
  MISC_FEATURE (4)..(4): Ala, Norval, Val, Norleu or Gly
  MISC_FEATURE (5)..(5): Ala or Thr
  MISC_FEATURE (6)..(6): Ala, Phe, Tyr or naphthylalanine
  MISC_FEATURE (7)..(7): Thr or Ser
  MISC_FEATURE (8)..(8): Ala, Ser or Thr
  MISC_FEATURE (9)..(9): Ala, Norval, Val, Norleu, Asp or Glu
  MISC_FEATURE (10)..(10): Ala, Leu, Ile, Val, pentylglycine or Met
  MISC_FEATURE (11)..(11): Ala or Ser
  MISC_FEATURE (12)..(12): Ala or Lys
  MISC_FEATURE (13)..(13): Ala or Gln
  MISC_FEATURE (14)..(14): Ala, Leu, Ile, pentylglycine, Val or Met
  MISC_FEATURE (15)..(17): Ala or Glu
  MISC_FEATURE (19)..(19): Ala or Val
  MISC_FEATURE (20)..(20): Ala or Arg
  MISC_FEATURE (21)..(21): Ala, Leu or Lys-NH-R where R is Lys, Arg, C1-10 straight chain or branched alkanoyl or cycloalkylalkanoyl
  MISC_FEATURE (22)..(22): Phe, Tyr or naphthylalanine
  MISC_FEATURE (23)..(23): Ile, Val, Leu, pentylglycine, tert-butylglycine or Met
  MISC_FEATURE (24)..(24): Ala, Glu or Asp
  MISC_FEATURE (25)..(25): Ala, Trp, Phe, Tyr or naphthylalanine
  MISC_FEATURE (26)..(26): Ala or Leu
  MISC_FEATURE (27)..(27): Lys, Asn, Lys-NH-R or Ala where R is Lys, Arg, C1-10 straight chain or branched alkanoyl or cycloalkylalkanoyl
  MISC_FEATURE (28)..(28): Lys, Asn, Lys-NH-R or Ala where R is Lys, Arg, C1-10 straight chain or branched alkanoyl or cycloalkylalkanoyl and is optionally amidated
  MISC_FEATURE (29)..(30): Gly or absent and if present optionally amidated
  MISC_FEATURE (31)..(31): Pro, homoproline, 3Hyp, 4Hyp, thiproline, N-alkylglycine, N-alkylpentylglycine, N-alkylalanine or absent and if present optionally amidated
  MISC_FEATURE (32)..(33): Ser or absent and if present optionally amidated
  MISC_FEATURE (34)..(34): Gly or absent and if present optionally amidated
  MISC_FEATURE (35)..(35): Ala or absent and if present optionally amidated
  MISC_FEATURE (36)..(38): Pro, homoproline, 3Hyp, 4Hyp, thiproline, N-alkylglycine, N-alkylpentylglycine, N-alkylalanine or absent and if present optionally amidated
  MISC_FEATURE (39)..(39): Ser, Tyr or absent and if present optionally amidated

SEQ ID NO: 21 - protein, 39 aa, Artificial Sequence
  Exendin analog
  MISC_FEATURE (1)..(1): His, Arg or Tyr
  MISC_FEATURE (2)..(2): Ser, Gly, Ala or Thr
  MISC_FEATURE (3)..(3): Asp or Glu
  MISC_FEATURE (6)..(6): Phe, Tyr or naphthylalanine
  MISC_FEATURE (7)..(7): Thr or Ser
  MISC_FEATURE (8)..(8): Ser or Thr
  MISC_FEATURE (9)..(9): Asp or Glu
  MISC_FEATURE (10)..(10): Leu, Ile, Val, pentylglycine or Met
  MISC_FEATURE (14)..(14): Leu, Ile, pentylglycine, Val or Met
  MISC_FEATURE (22)..(22): Phe, Tyr or naphthylalanine
  MISC_FEATURE (23)..(23): Ile, Val, Leu, pentylglycine, tert-butylglycine or Met
  MISC_FEATURE (24)..(24): Glu or Asp
  MISC_FEATURE (25)..(25): Trp, Phe, Tyr or naphthylalanine
  MISC_FEATURE (31)..(31): Pro, homoproline, 3Hyp, 4Hyp, thioproline, N-alkylglycine, N-alkylpentylglycine or N-alkylalanine
  MISC_FEATURE (36)..(38): Pro, homoproline, 3Hyp, 4Hyp, thioproline, N-alkylglycine, N-alkylpentylglycine or N-alkylalanine
  MISC_FEATURE (39)..(39): Ser, Thr or Tyr and optionally amidated
XXXGTXXXXXSKQXEEEAVRLXXXXLKNGGXSSGAXXXX

SEQ ID NO: 22 - protein, 39 aa, Artificial Sequence
  Exendin analog
  MISC_FEATURE (1)..(1): His, Arg, Tyr, 4-imidazopropionyl
  MISC_FEATURE (2)..(2): Ser, Gly, Ala or Thr
  MISC_FEATURE (3)..(3): Asp or Glu
  MISC_FEATURE (6)..(6): Phe, Tyr or naphthylalanine
  MISC_FEATURE (7)..(8): Thr or Ser
  MISC_FEATURE (9)..(9): Asp or Glu
  MISC_FEATURE (10)..(10): Leu, Ile, Val, pentylglycine or Met
  MISC_FEATURE (14)..(14): Leu, Ile, pentylglycine, Val or Met
  MISC_FEATURE (22)..(22): Phe, Tyr or naphthylalanine
  MISC_FEATURE (23)..(23): Ile, Val, Leu, pentylglycine, tert-butylglycine or Met
  MISC_FEATURE (24)..(24): Glu or Asp
  MISC_FEATURE (25)..(25): Trp, Phe, Tyr, or naphthylalanine
  MISC_FEATURE (27)..(28): Lys, Asn or Lys-NH-R where R is Lys, Arg, C1-C10 straight chain or branched alkanoyl or cycloalkylalkanoyl
  MISC_FEATURE (31)..(31): Pro, homoproline, 3Hyp, 4Hyp, thioproline, N-alkylglycine, N-alkylpentylglycine or N-alkylalanine
  MISC_FEATURE (36)..(38): Pro, homoproline, 3Hyp, 4Hyp, thioproline, N-alkylglycine, N-alkylpentylglycine or N-alkylalanine
  MISC_FEATURE (39)..(39): Ser, Thr or Tyr and is optionally amidated
XXXGTXXXXXSKQXEEEAVRLXXXXLXXGGXSSGAXXXX

SEQ ID NO: 23 - protein, 30 aa, Artificial Sequence; identical to SEQ ID NO: 9
  Exendin analog
  MOD_RES (30)...(30): AMIDATION

SEQ ID NO: 24 - protein, 28 aa, Artificial Sequence
  Exendin analog
  MOD_RES (28)...(28): AMIDATION
HGEGTFTSDLSKQMEEEAVRLFIEWLKN

SEQ ID NO: 25 - protein, 28 aa, Artificial Sequence
  Exendin analog
  MOD_RES (28)...(28): AMIDATION
HGEGTFTSDLSKQLEEEAVRLFIEFLKN

SEQ ID NO: 26 - protein, 28 aa, Artificial Sequence
  Exendin analog
  MOD_RES (28)...(28): AMIDATION
HAEGTFTSDLSKQLEEEAVRLFIEFLKN

SEQ ID NO: 27 - protein, 28 aa, Artificial Sequence
  Exendin analog
  MOD_RES (28)...(28): AMIDATION
HGEGAFTSDLSKQLEEEAVRLFIEFLKN

SEQ ID NO: 28 - protein, 28 aa, Artificial Sequence
  Exendin analog
  MOD_RES (28)...(28): AMIDATION
HGEGTATSDLSKQLEEEAVRLFIEFLKN

SEQ ID NO: 29 - protein, 28 aa, Artificial Sequence
  Exendin analog
  MOD_RES (28)...(28): AMIDATION
HGEGTFTADLSKQLEEEAVRLFIEFLKN

SEQ ID NO: 30 - protein, 28 aa, Artificial Sequence
  Exendin analog
  MOD_RES (28)...(28): AMIDATION
HGEGTFTSDASKQLEEEAVRLFIEFLKN

SEQ ID NO: 31 - protein, 28 aa, Artificial Sequence
  Exendin analog
  MOD_RES (28)...(28): AMIDATION
HGEGTFTSDLAKQLEEEAVRLFIEFLKN

SEQ ID NO: 32 - protein, 28 aa, Artificial Sequence
  Exendin analog
  MOD-RES (28)...(28): AMIDATION
HGEGTFTSDLSAQLEEEAVRLFIEFLKN

SEQ ID NO: 33 - protein, 28 aa, Artificial Sequence
  Exendin analog
  MOD_RES (28)...(28): AMIDATION
HGEGTFTSDLSKALEEEAVRLFIEFLKN

SEQ ID NO: 34 - protein, 28 aa, Artificial Sequence
  Exendin analog
  MOD_RES (28)...(28): AMIDATION
HGEGTFTSDLSKQAEEEAVRLFIEFLKN

SEQ ID NO: 35 - protein, 28 aa, Artificial Sequence
  Exendin analog
  MOD_RES (28)...(28): AMIDATION
HGEGTFTSDLSKQLAEEAVRLFIEFLKN

SEQ ID NO: 36 - protein, 28 aa, Artificial Sequence
  Exendin analog
  MOD_RES (28)...(28): AMIDATION
HGEGTFTSDLSKQLEAEAVRLFIEFLKN

SEQ ID NO: 37 - protein, 28 aa, Artificial Sequence
  Exendin analog
  MOD_RES (28)...(28): AMIDATION
HGEGTFTSDLSKQLEEAAVRLFIEFLKN

SEQ ID NO: 38 - protein, 28 aa, Artificial Sequence
  artificially synthesized sequence of novel exendin agonist compound
  AMIDATION (28)...(28): amidated Asn (Asparaginamide)
HGEGTFTSDLSKQLEEEAARLFIEFLKN

SEQ ID NO: 39 - protein, 28 aa, Artificial Sequence
  Exendin analog
  MOD_RES (28)...(28): AMIDATION
HGEGTFTSDLSKQLEEEAVALFIEFLKN

SEQ ID NO: 40 - protein, 28 aa, Artificial Sequence
  Exendin analog
  MOD_RES (28)...(28): AMIDATION
HGEGTFTSDLSKQLEEEAVRAFIEFLKN

SEQ ID NO: 41 - protein, 28 aa, Artificial Sequence
  Exendin analog
  MOD_RES (28)...(28): AMIDATION
HGEGTFTSDLSKQLEEEAVRLFIAFLKN

SEQ ID NO: 42 - protein, 28 aa, Artificial Sequence
  Exendin analog
  MOD_RES (28)...(28): AMIDATION
HGEGTFTSDLSKQLEEEAVRLFIEALKN

SEQ ID NO: 43 - protein, 28 aa, Artificial Sequence
  Exendin analog
  MOD-RES (28)...(28): AMIDATION
HGEGTFTSDLSKQLEEEAVRLFIEFAKN

SEQ ID NO: 44 - protein, 28 aa, Artificial Sequence
  Exendin analog
  MOD_RES (28)...(28): AMIDATION
HGEGTFTSDLSKQLEEEAVRLFIEFLAN

SEQ ID NO: 45 - protein, 28 aa, Artificial Sequence
  Exendin analog
  MOD-RES (28)...(28): AMIDATION
HGEGTFTSDLSKQLEEEAVRLFIEFLKA

SEQ ID NO: 46 - protein, 38 aa, Artificial Sequence
  Exendin analog
  MOD_RES (38)...(38): AMIDATION
HGEGTFTSDLSKQMEEEAVRLFIEWLKNGGPSSGAPPP

SEQ ID NO: 47 - protein, 38 aa, Artificial Sequence
  Exendin analog
  MOD_RES (38)...(38): AMIDATION
HGEGTFTSDLSKQLEEEAVRLFIEFLKNGGPSSGAPPP

SEQ ID NO: 48 - protein, 37 aa, Artificial Sequence
  Exendin analog
  MOD_RES (37)...(37): AMIDATION
HGEGTFTSDLSKQMEEEAVRLFIEWLKNGGPSSGAPP

SEQ ID NO: 49 - protein, 37 aa, Artificial Sequence
  Exendin analog
  MOD_RES (37)...(37): AMIDATION
HGEGTFTSDLSKQLEEEAVRLFIEFLKNGGPSSGAPP

SEQ ID NO: 50 - protein, 36 aa, Artificial Sequence
  Exendin analog
  MOD_RES (36)...(36): AMIDATION
HGEGTFTSDLSKQMEEEAVRLFIEWLKNGGPSSGAP

SEQ ID NO: 51 - protein, 36 aa, Artificial Sequence
  Exendin analog
  MOD_RES (36)...(36): AMIDATION
HGEGTFTSDLSKQLEEEAVRLFIEFLKNGGPSSGAP

SEQ ID NO: 52 - protein, 35 aa, Artificial Sequence
  Exendin analog
  MOD_RES (35)...(35): AMIDATION
HGEGTFTSDLSKQMEEEAVRLFIEWLKNGGPSSGA

SEQ ID NO: 53 - protein, 35 aa, Artificial Sequence
  Exendin analog
  MOD_RES (35)...(35): AMIDATION
HGEGTFTSDLSKQLEEEAVRLFIEFLKNGGPSSGA

SEQ ID NO: 54 - protein, 34 aa, Artificial Sequence
  Exendin analog
  MOD_RES (34)...(34): AMIDATION
HGEGTFTSDLSKQMEEEAVRLFIEWLKNGGPSSG

SEQ ID NO: 55 - protein, 34 aa, Artificial Sequence
  Exendin analog
  MOD_RES (34)...(34): AMIDATION
HGEGTFTSDLSKQLEEEAVRLFIEFLKNGGPSSG

SEQ ID NO: 56 - protein, 33 aa, Artificial Sequence
  Exendin analog
  MOD_RES (33)...(33): AMIDATION
HGEGTFTSDLSKQMEEEAVRLFIEWLKNGGPSS

SEQ ID NO: 57 - protein, 33 aa, Artificial Sequence
  Exendin analog
  MOD_RES (33)...(33): AMIDATION
HGEGTFTSDLSKQLEEEAVRLFIEFLKNGGPSS

SEQ ID NO: 58 - protein, 32 aa, Artificial Sequence
  Exendin analog
  MOD_RES (32)...(32): AMIDATION
HGEGTFTSDLSKQMEEEAVRLFIEWLKNGGPS

SEQ ID NO: 59 - protein, 32 aa, Artificial Sequence
  Exendin analog
  MOD_RES (32)...(32): AMIDATION
HGEGTFTSDLSKQLEEEAVRLFIEFLKNGGPS

SEQ ID NO: 60 - protein, 31 aa, Artificial Sequence
  Exendin analog
  MOD_RES (31)...(31): AMIDATION
HGEGTFTSDLSKQMEEEAVRLFIEWLKNGGP

SEQ ID NO: 61 - protein, 31 aa, Artificial Sequence
  Exendin analog
  MOD_RES (31)...(31): AMIDATION
HGEGTFTSDLSKQLEEEAVRLFIEFLKNGGP

SEQ ID NO: 62 - protein, 30 aa, Artificial Sequence
  Exendin analog
  MOD_RES (30)...(30): AMIDATION
HGEGTFTSDLSKQLEEEAVRLFIEFLKNGG

SEQ ID NO: 63 - protein, 29 aa, Artificial Sequence
  Exendin analog
  MOD_RES (29)...(29): AMIDATION
HGEGTFTSDLSKQMEEEAVRLFIEWLKNG

SEQ ID NO: 64 - protein, 29 aa, Artificial Sequence
  Exendin analog
  MOD_RES (29)...(29): AMIDATION
HGEGTFTSDLSKQLEEEAVRLFIEFLKNG

SEQ ID NO: 65 - protein, 38 aa, Artificial Sequence
  Exendin analog
  MISC_FEATURE (31)...(31): thioproline
  MISC_FEATURE (36)...(38): thioproline
  MOD_RES (38)...(38): AMIDATION
HGEGTFTSDLSKQMEEEAVRLFIEWLKNGGXSSGAXXX

SEQ ID NO: 66 - protein, 38 aa, Artificial Sequence
  Exendin analog
  MISC_FEATURE (36)...(38): thioproline
  MOD_RES (38)...(38): AMIDATION
HGEGTFTSDLSKQMEEEAVRLFIEWLKNGGPSSGAXXX

SEQ ID NO: 67 - protein, 37 aa, Artificial Sequence
  Exendin analog
  MOD_RES (31)...(31): N-methyl ala.
  MOD_RES (37)...(37): AMIDATION
HGEGTFTSDLSKQMEEEAVRLFIEWLKNGGASSGAPP

SEQ ID NO: 68 - protein, 37 aa, Artificial Sequence
  Exendin analog
  MOD_RES (31)...(31): N-methyl ala
  MOD_RES (36)...(37): N-methyl ala
  MOD_RES (37)...(37): AMIDATION
HGEGTFTSDLSKQMEEEAVRLFIEWLKNGGASSGAAA

SEQ ID NO: 69 - protein, 37 aa, Artificial Sequence
  Exendin analog
  MISC_FEATURE (31)...(31): homoproline
  MISC_FEATURE (36)...(37): homoproline
  MOD_RES (37)...(37): AMIDATION
HGEGTFTSDLSKQMEEEAVRLFIEWLKNGGXSSGAXX

SEQ ID NO: 70 - protein, 36 aa, Artificial Sequence
  Exendin analog
  MISC_FEATURE (31)...(31): homoproline
  MISC_FEATURE (36)...(36): homoproline.
  MOD_RES (36)...(36): AMIDATION
HGEGTFTSDLSKQMEEEAVRLFIEWLKNGGXSSGAX

SEQ ID NO: 71 - protein, 35 aa, Artificial Sequence
  Exendin analog
  MOD_RES (35)...(35): AMIDATION
RGEGTFTSDLSKQMEEEAVRLFIEWLKNGGPSSGA

SEQ ID NO: 72 - protein, 30 aa, Artificial Sequence
  Exendin analog
  MOD_RES (30)...(30): AMIDATION
HGDGTFTSDLSKQMEEEAVRLFIEWLKNGG

SEQ ID NO: 73 - protein, 28 aa, Artificial Sequence
  Exendin analog
  MISC_FEATURE (6)...(6): naphthylalanine
  MOD_RES (28)...(28): AMIDATION
HGEGTXTSDLSKQLEEEAVRLFIEFLKN

SEQ ID NO: 74 - protein, 28 aa, Artificial Sequence
  Exendin analog
  MOD_RES (28)...(28): AMIDATION
HGEGTFSSDLSKQMEEEAVRLFIEWLKN

SEQ ID NO: 75 - protein, 28 aa, Artificial Sequence
  Exendin analog
  MOD_RES (28)...(28): AMIDATION
HGEGTFSTDLSKQMEEEAVRLFIEWLKN

SEQ ID NO: 76 - protein, 28 aa, Artificial Sequence
  Exendin analog
  MOD_RES (28)...(28): AMIDATON
HGEGTFTSELSKQMAEEAVRLFIEWLKN

SEQ ID NO: 77 - protein, 28 aa, Artificial Sequence
  Exendin analog
  MISC_FEATURE (10)...(10): pentylglycine
  MOD_RES (28)...(28): AMIDATION
HGEGTFTSDXSKQLEEEAVRLFIEFLKN

SEQ ID NO: 78 - protein, 28 aa, Artificial Sequence
  Exendin analog
  MISC_FEATURE (22)...(22): naphthylalanine
  MOD_RES (28)...(28): AMIDATION
HGEGTFTSDLSKQLEEEAVRLXIEFLKN

SEQ ID NO: 79 - protein, 28 aa, Artificial Sequence
  Exendin analog
  MISC_FEATURE (23)...(23): tert-butylglycine
  MOD_RES (28)...(28): AMIDATION
HGEGTFTSDLSKQMEEEAVRLFXEWLKN

SEQ ID NO: 80 - protein, 28 aa, Artificial Sequence
  Exendin analog
  MOD_RES (28)...(28): AMIDATION
HGEGTFTSDLSKQLEEEAVRLFIDFLKN

SEQ ID NO: 81 - protein, 33 aa, Artificial Sequence
  Exendin analog
  MOD_RES (33)...(33): AMIDATION
HGEGTFTSDASKQLEEEAVRLFIEFLKNGGPSS

SEQ ID NO: 82 - protein, 29 aa, Artificial Sequence
  Exendin analog
  MOD_RES (29)...(29): AMIDATON
HGEGTFTSDASKQMEEEAVRLFIEWLKNG

SEQ ID NO: 83 - protein, 37 aa, Artificial Sequence
  artificially synthesized sequence of novel exendin agonist compound
  MISC_FEATURE (31)...(31): homoproline
  MISC_FEATURE (36)...(37): homoproline
  MOD_RES (37)...(37): AMIDATION
HGEGTFTSDASKQMEEEAVRLFIEWLKNGGXSSGAXX

SEQ ID NO: 84 - protein, 27 aa, Artificial Sequence
  Exendin analog
  MOD_RES (1)...(1): 4-imidazolylpropionyl-Gly
  MOD_RES (26)...(26): Lys-NH(epsilon)octanoyl.
  MOD_RES (27)...(27): AMIDATION
GEGTFTSDLSKQMEEEAVRLFIEWLKN

SEQ ID NO: 85 - protein, 27 aa, Artificial Sequence
  Exendin analog
  MOD_RES (1)...(1): 4-imidazolylpropionyl-Gly
  MOD_RES (26)...(26): Lys-NH(epsilon)octanoyl.
  MOD_RES (27)...(27): AMIDATION
GEGTFTSDLSKQLEEEAVRLFIEFLKN

SEQ ID NO: 86 - protein, 29 aa, Artificial Sequence
  Exendin analog
  MOD_RES (1)...(1): 4-imidazolylpropionyl-Gly
  MOD_RES (26)...(26): Lys-NH(epsilon)octanoyl.
  MOD_RES (29)...(29): AMIDATION
GEGTFTSDLSKQMEEEAVRLFIEWLKNGG

SEQ ID NO: 87 - protein, 29 aa, Artificial Sequence
  Exendin analog
  MOD_RES (1)...(1): 4-imidazolylpropionyl-Gly
  MOD_RES (26)...(26): Lys-NH(epsilon)octanoyl.
  MOD_RES (29)...(29): AMIDATION
GEGTFTSDLSKQLEEEAVRLFIEFLKNGG

SEQ ID NO: 88 - protein, 27 aa, Artificial Sequence
  Exendin analog
  MOD_RES (1)...(1): 4-imidazolylpropionyl-Gly
  MOD_RES (27)...(27): Lys-NH(epsilon)octanoyl.
  MOD_RES (27)...(27): AMIDATION
GEGTFTSDLSKQMEEEAVRLFIEWLNK

SEQ ID NO: 89 - protein, 27 aa, Artificial Sequence
  Exendin analog
  MOD_RES (1)...(1): 4-imidazolylpropionyl-Gly
  MOD_RES (27)...(27): Lys-NH(epsilon)octanoyl.
  MOD_RES (27)...(27): AMIDATION
GEGTFTSDLSKQLEEEAVRLFIEFLNK

SEQ ID NO: 90 - protein, 29 aa, Artificial Sequence
  Exendin analog
  MOD_RES (1)...(1): 4-imidazolylpropionyl-Gly
  MOD_RES (27..(27): Lys-NH(epsilon)octanoyl.
  MOD_RES (29)...(29): AMIDTION
GEGTFTSDLSKQMEEEAVRLFIEWLNKGG

SEQ ID NO: 91 - protein, 29 aa, Artificial Sequence
  Exendin analog
  MOD-RES (1)...(1): 4-imidazolylpropionyl-Gly
  MOD_RES (27)...(27): Lys-NH(epsilon)octanoyl.
  MOD_RES (29)...(29): AMIDATION
GEGTFTSDLSKQLEEEAVRLFIEFLNKGG

SEQ ID NO: 92 - protein, 27 aa, Artificial Sequence
  Exendin analog
  MOD_RES (27)...(27): AMIDATION
  MOD_RES (1)...(1): 4-imidazolylpropionyl-Gly
  MOD_RES (26)...(26): Lys-NH(epsilon)octanoyl
XEGTFTSALSKQMEEEAVRLFIEWLXN

SEQ ID NO: 93 - protein, 27 aa, Artificial Sequence
  Exendin analog
  MOD_RES (27)...(27): AMIDATION
  MOD_RES (1)...(1): 4-imidazolylpropionyl-Gly
  MOD_RES (26)...(26): Lys-NH(epsilon)octanoyl
XEGTFTSALSKQLEEEAVRLFIEFLXN

SEQ ID NO: 94 - protein, 29 aa, Artificial Sequence
  Exendin analog
  MOD_RES (29)...(29): AMIDATION
  MOD_RES (1)...(1): 4-imidazolylpropionyl-Gly
  MOD_RES (26),,,(26): Lys-NH(epsilon)octanoyl
XEGTFTSALSKQMEEEAVRLFIEWLXNGG

SEQ ID NO: 95 - protein, 29 aa, Artificial Sequence
  Exendin analog
  MOD_RES (29)...(29): AMIDATION
  MOD_RES (1)...(1): 4-imidazolylpropionyl-Gly
  MOD_RES (26)...(26): Lys-NH(epsilon)octanoyl
XEGTFTSALSKQLEEEAVRLFIEFLXNGG

SEQ ID NO: 96 - protein, 27 aa, Artificial Sequence
  Exendin analog
  MOD_RES (27)...(27): AMIDATION
  MOD_RES (1)...(1): 4-imidazolylpropionyl-Gly
  MOD_RES (27)...(27): Lys-NH(epsilon)octanoyl
XEGTFTSALSKQMEEEAVRLFIEWLNX

SEQ ID NO: 97 - protein, 27 aa, Artificial Sequence
  Exendin analog
  MOD_RES (27)...(27): AMIDATION
  MOD_RES (1)...(1): 4-imidazolylpropionyl-Gly
  MOD_RES (27)...(27): Lys-NH(epsilon)octanoyl
XEGTFTSALSKQLEEEAVRLFIEFLNX

SEQ ID NO: 98 - protein, 29 aa, Artificial Sequence
  Exendin analog
  MOD_RES (29)...(29): AMIDATION
  MOD_RES (1)...(1): 4-imidazolylpropionyl-Gly
  MOD_RES (27)...(27): Lys-NH(epsilon)octanoyl
XEGTFTSALSKQMEEEAVRLFIEWLNXGG

SEQ ID NO: 99 - protein, 29 aa, Artificial Sequence
  Exendin analog
  MOD_RES (29)...(29): AMIDATION
  MOD_RES (1),,,(1): 4-imidazolylpropionyl-Gly
  MOD_RES (27),,,(27): Lys-NH(epsilon)octanoyl
XEGTFTSALSKQLEEEAVRLFIEFLNXGG

SEQ ID NO: 100 - protein, 28 aa, Artificial Sequence
  Exendin analog
  MOD_RES (28)...(28): AMIDATION
  MOD_RES (27)...(27): Lys-NH(epsilon)octanoyl
AGEGTFTSDLSKQMEEEAVRLFIEWLXN

SEQ ID NO: 101 - protein, 28 aa, Artificial Sequence
  Exendin analog
  MOD_RES (28)...(28): AMIDATION
  MOD_RES (27)...(27): Lys-NH(epsilon)octanoyl
AGEGTFTSDLSKQLEEEAVRLFIEFLXN

SEQ ID NO: 102 - protein, 30 aa, Artificial Sequence
  Exendin analog
  MOD_RES (30)...(30): AMIDATION
  MOD_RES (27)...(27): Lys-NH(epsilon)octanoyl
AGEGTFTSDLSKQMEEEAVRLFIEWLXNGG

SEQ ID NO: 103 - protein, 30 aa, Artificial Sequence
  Exendin analog
  MOD_RES (30)...(30): AMIDATION
  MOD_RES (27)...(27): Lys-NH(epsilon)octanoyl
AGEGTFTSDLSKQLEEEAVRLFIEFLXNGG

SEQ ID NO: 104 - protein, 28 aa, Artificial Sequence
  Exendin analog
  MOD_RES (28)...(28): AMIDATION
  MOD_RES (27)...(27): Lys-NH(epsilon)octanoyl
AGEGTFTSDLSKQMEEEAVRLFIEWLNX

SEQ ID NO: 105 - protein, 28 aa, Artificial Sequence
  Exendin analog
  MOD_RES (28)...(28): AMIDATION
  MOD_RES (27)...(27): Lys-NH(epsilon)octanoyl
AGEGTFTSDLSKQLEEEAVRLFIEFLNX

SEQ ID NO: 106 - protein, 30 aa, Artificial Sequence
  Exendin analog
  MOD_RES (30)...(30): AMIDATION
  MOD_RES (27)...(27): Lys-NH(epsilon)octanoyl
AGEGTFTSDLSKQMEEEAVRLFIEWLNXGG

SEQ ID NO: 107 - protein, 30 aa, Artificial Sequence
  Exendin analog
  MOD_RES (30)...(30): AMIDATION
  MOD_RES (27)...(27): Lys-NH(epsilon)octanoyl
AGEGTFTSDLSKQLEEEAVRLFIEFLNXGG

SEQ ID NO: 108 - protein, 39 aa, Artificial Sequence; identical to SEQ ID NO: 12
  Exendin analog
  MOD-RES (39)...(39): AMIDATION

SEQ ID NO: 109 - protein, 39 aa, Artificial Sequence
  Exendin analog
  MOD-RES (39)...(39): AMIDATION
HGEGTFTSDLSKQLEEEAVRLFIEWLKNGGPSSGAPPPS

SEQ ID NO: 110 - protein, 39 aa, Artificial Sequence
  Exendin analog
  MOD-RES (39)...(39): AMIDATION
HGEGTFTSDLSKQMEEEAVRLFIEFLKNGGPSSGAPPPS

SEQ ID NO: 111 - protein, 39 aa, Artificial Sequence
  Exendin analog
  MOD-RES (39)...(39): AMIDATION
YGEGTFTSDLSKQMEEEAVRLFIEWLKNGGPSSGAPPPS

SEQ ID NO: 112 - protein, 39 aa, Artificial Sequence
  Exendin analog
  MOD-RES (39)...(39): AMIDATION
HGEGTFTSDLSKQMEEEAVRLFIEWLKNGGPSSGAPPPY

SEQ ID NO: 113 - protein, 39 aa, Artificial Sequence
  Exendin analog
  MOD-RES (39)...(39): AMIDATION
HGDGTFTSDLSKQMEEEAVRLFIEWLKNGGPSSGAPPPS

SEQ ID NO: 114 - protein, 39 aa, Artificial Sequence
  Exendin analog
  MOD_RES (6)...(6): napthylalanine
  MOD-RES (39)...(39): AMIDATION
HGEGTXTSDLSKQMEEEAVRLFIEWLKNGGPSSGAPPPS

SEQ ID NO: 115 - protein, 39 aa, Artificial Sequence
  Exendin analog
  MOD-RES (39)...(39): AMIDATION
HGEGTFSSDLSKQMEEEAVRLFIEWLKNGGPSSGAPPPS

SEQ ID NO: 116 - protein, 39 aa, Artificial Sequence
  Exendin analog
  MOD-RES (39)...(39): AMIDATION
HGEGTFSTDLSKQMEEEAVRLFIEWLKNGGPSSGAPPPS

SEQ ID NO: 117 - protein, 39 aa, Artificial Sequence
  Exendin analog
  MOD-RES (39)...(39): AMIDATION
HGEGTFTTDLSKQMEEEAVRLFIEWLKNGGPSSGAPPPS

SEQ ID NO: 118 - protein, 39 aa, Artificial Sequence
  Exendin analog
  MOD-RES (39)...(39): AMIDATION
HGEGTFTSELSKQMEEEAVRLFIEWLKNGGPSSGAPPPS

SEQ ID NO: 119 - protein, 39 aa, Artificial Sequence
  Exendin analog
  MOD_RES (10)...(10): pentylglycine
  MOD-RES (39)...(39): AMIDATION
HGEGTFTSDXSKQMEEEAVRLFIEWLKNGGPSSGAPPPS

SEQ ID NO: 120 - protein, 39 aa, Artificial Sequence
  Exendin analog
  MOD_RES (10)...(10): pentylglycine
  MOD-RES (39)...(39): AMIDATION
HGEGTFTSDXSKQLEEEAVRLFIEFLKNGGPSSGAPPPS

SEQ ID NO: 121 - protein, 39 aa, Artificial Sequence
  Exendin analog
  MOD_RES (14)...(14): pentylglycine
  MOD-RES (39)...(39): AMIDATION
HGEGTFTSDLSKQXEEEAVRLFIEWLKNGGPSSGAPPPS

SEQ ID NO: 122 - protein, 39 aa, Artificial Sequence; identical to SEQ ID NO: 12
  Exendin analog
  MOD-RES (39)...(39): AMIDATION
  MOD_RES (14)...(14): pentylglycine

SEQ ID NO: 123 - protein, 39 aa, Artificial Sequence
  Exendin analog
  MOD_RES (22)..(22): napthylalanine
  MOD-RES (39)...(39): AMIDATION
HGEGTFTSDLSKQMEEEAVRLXIEWLKNGGPSSGAPPPS

SEQ ID NO: 124 - protein, 39 aa, Artificial Sequence
  Exendin analog
  MOD-RES (39)...(39): AMIDATION
HGEGTFTSDLSKQMEEEAVRLFVEWLKNGGPSSGAPPPS

SEQ ID NO: 125 - protein, 39 aa, Artificial Sequence
  Exendin analog
  MOD-RES (39)...(39): AMIDATION
HGEGTFTSDLSKQLEEEAVRLFVEFLKNGGPSSGAPPPS

SEQ ID NO: 126 - protein, 39 aa, Artificial Sequence
  Exendin analog
  MOD_RES (23)...(23): tert-butylglycine
  MOD-RES (39)...(39): AMIDATION
HGEGTFTSDLSKQMEEEAVRLFXEWLKNGGPSSGAPPPS

SEQ ID NO: 127 - protein, 39 aa, Artificial Sequence
  Exendin analog
  MOD_RES (23)...(23): tert-butylglycine
  MOD-RES (39)...(39): AMIDATION
HGEGTFTSDLSKQLEEEAVRLFXEFLKNGGPSSGAPPPS

SEQ ID NO: 128 - protein, 39 aa, Artificial Sequence
  Exendin analog
  MOD-RES (39)...(39): AMIDATION
HGEGTFTSDLSKQMEEEAVRLFIDWLKNGGPSSGAPPPS

SEQ ID NO: 129 - protein, 39 aa, Artificial Sequence; identical to SEQ ID NO: 110
  Exendin analog
  MOD-RES (39)...(39): AMIDATION

SEQ ID NO: 130 - protein, 39 aa, Artificial Sequence
  Exendin analog
  MOD_RES (31)...(31): thioproline
  MOD_RES (36)..(38): thioproline
  MOD-RES (39)...(39): AMIDATION
HGEGTFTSDLSKQMEEEAVRLFIEWLKNGGXSSGAXXXS

SEQ ID NO: 131 - protein, 39 aa, Artificial Sequence
  Exendin analog
  MOD_RES (36)..(38): thioproline
  MOD-RES (39)...(39): AMIDATION
HGEGTFTSDLSKQMEEEAVRLFIEWLKNGGPSSGAXXXS

SEQ ID NO: 132 - protein, 39 aa, Artificial Sequence; identical to SEQ ID NO: 130
  Exendin analog
  MOD_RES (31)...(31): homoproline
  MOD_RES (36)..(38): homoproline
  MOD-RES (39)...(39): AMIDATION

SEQ ID NO: 133 - protein, 39 aa, Artificial Sequence; identical to SEQ ID NO: 131
  Exendin analog
  MOD_RES (36)..(38): homoproline
  MOD-RES (39)...(39): AMIDATION

SEQ ID NO: 134 - protein, 39 aa, Artificial Sequence
  Exendin analog
  MOD_RES (31)...(31): thioproline
  MOD_RES (36)..(38): thioproline
  MOD-RES (39)...(39): AMIDATION
HGEGTFTSDLSKQLEEEAVRLFIEFLKNGGXSSGAXXXS

SEQ ID NO: 135 - protein, 39 aa, Artificial Sequence; identical to SEQ ID NO: 134
  Exendin analog
  MOD_RES (31)...(31): homoproline
  MOD_RES (36)..(38): homoproline
  MOD-RES (39)...(39): AMIDATION

SEQ ID NO: 136 - protein, 39 aa, Artificial Sequence; identical to SEQ ID NO: 130
  Exendin analog
  MOD_RES (31)...(31): N-methylalanine
  MOD_RES (36)..(38): N-methylalanine
  MOD-RES (39)...(39): AMIDATION

SEQ ID NO: 137 - protein, 39 aa, Artificial Sequence; identical to SEQ ID NO: 131
  Exendin analog
  MOD_RES (36)..(38): N-methylalanine
  MOD-RES (39)...(39): AMIDATION

SEQ ID NO: 138 - protein, 39 aa, Artificial Sequence; identical to SEQ ID NO: 134
  Exendin analog
  MOD_RES (31)...(31): N-methylalanine
  MOD_RES (36)..(38): N-methylalanine
  MOD-RES (39)...(39): AMIDATION

SEQ ID NO: 139 - protein, 39 aa, Artificial Sequence
  Exendin analog
  MOD_RES (1)...(1): 4-Imidazolylpropionyl
  MOD_RES (27)...(27): Lys-NH(epsilon) octanoyl
  MOD-RES (39)...(39): AMIDATION
XGEGTFTSDLSKQMEEEAVRLFIEWLKNGGPSSGAPPPS

SEQ ID NO: 140 - protein, 39 aa, Artificial Sequence
  Exendin analog
  MOD_RES (1)...(1): 4-Imidazolylpropionyl
  MOD_RES (27)...(27): Lys-NH(epsilon) octanoyl
  MOD-RES (39)...(39): AMIDATION
XGEGTFTSDLSKQLEEEAVRLFIEFLKNGGPSSGAPPPS

SEQ ID NO: 141 - protein, 39 aa, Artificial Sequence
  Exendin analog
  MOD_RES (1)...(1): 4-Imidazolylpropionyl
  MOD_RES (28)...(28): Lys-NH(epsilon) octanoyl
  MOD-RES (39)...(39): AMIDATION
XGEGTFTSDLSKQMEEEAVRLFIEWLNKGGPSSGAPPPS

SEQ ID NO: 142 - protein, 39 aa, Artificial Sequence
  Exendin analog
  MOD_RES (1)...(1): 4-Imidazolylpropionyl
  MOD_RES (28)...(28): Lys-NH(epsilon) octanoyl
  MOD-RES (39)...(39): AMIDATION
XGEGTFTSDLSKQLEEEAVRLFIEFLNKGGPSSGAPPPS